European Patent Specification EP 3 772 543 B1, published September 27, 2023. Title: Method for diagnosing breast cancer. Applicant: Albert-Ludwigs-Universitaet Freiburg. The sequence listing filed with the application follows.

SEQUENCE LISTING (52 sequences)

SEQ ID NO: 1 - RNA, 22 nt, Caenorhabditis elegans
ucaccggguguaaaucagcuug

SEQ ID NO: 2 - RNA, 21 nt, Arabidopsis thaliana
uuuggauugaagggagcucua

SEQ ID NO: 3 - RNA, 22 nt, Homo sapiens
uagcagcacguaaauauuggcg

SEQ ID NO: 4 - RNA, 23 nt, Homo sapiens
caaagugcuuacagugcagguag

SEQ ID NO: 5 - RNA, 21 nt, Homo sapiens
uucaaguaauucaggauaggu

SEQ ID NO: 6 - RNA, 23 nt, Homo sapiens
agcagcauuguacagggcuauca

SEQ ID NO: 7 - RNA, 22 nt, Homo sapiens
ucccugagacccuaacuuguga

SEQ ID NO: 8 - RNA, 22 nt, Homo sapiens
uguaacagcaacuccaugugga

SEQ ID NO: 9 - RNA, 21 nt, Homo sapiens
agcuacaucuggcuacugggu

SEQ ID NO: 10 - RNA, 23 nt, Homo sapiens
ugaggggcagagagcgagacuuu

SEQ ID NO: 11 - RNA, 22 nt, Homo sapiens
cagcagcaauucauguuuugaa

SEQ ID NO: 12 - RNA, 22 nt, Homo sapiens
uacccauugcauaucggaguug

SEQ ID NO: 13 - RNA, 22 nt, Homo sapiens
ugagguaguagguuguauaguu

SEQ ID NO: 14 - RNA, 22 nt, Homo sapiens
agagguaguagguugcauaguu

SEQ ID NO: 15 - RNA, 22 nt, Homo sapiens
ugagguaggagguuguauaguu

SEQ ID NO: 16 - RNA, 22 nt, Homo sapiens
ugagguaguagauuguauaguu

SEQ ID NO: 17 - RNA, 22 nt, Homo sapiens
ugagguaguaguuugugcuguu

SEQ ID NO: 18 - DNA, 19 bp, Artificial Sequence
  sense primer for cel-miR39-3p
gtcaccgggtgtaaatcag

SEQ ID NO: 19 - DNA, 26 bp, Artificial Sequence
  antisense primer for cel-miR39-3p
ggtccagtttttttttttttttcaag

SEQ ID NO: 20 - DNA, 18 bp, Artificial Sequence
  sense primer for ath-miR159a
gcgcagtttggattgaag

SEQ ID NO: 21 - DNA, 27 bp, Artificial Sequence
  antisense primer for ath-miR159a
aggtccagtttttttttttttttagag

SEQ ID NO: 22 - DNA, 17 bp, Artificial Sequence
  sense primer for hsa-miR16-5p
cgcagtagcagcacgta

SEQ ID NO: 23 - DNA, 24 bp, Artificial Sequence
  antisense primer for hsa-miR16-5p
cagtttttttttttttttcgccaa

SEQ ID NO: 24 - DNA, 20 bp, Artificial Sequence
  sense primer for hsa-miR17-5p
gcaaagtgcttacagtgcag

SEQ ID NO: 25 - DNA, 26 bp, Artificial Sequence
  antisense primer for hsa-miR17-5p
ggtccagtttttttttttttttctac

SEQ ID NO: 26 - DNA, 22 bp, Artificial Sequence
  sense primer for hsa-miR26b-5p
cgcagttcaagtaattcaggat

SEQ ID NO: 27 - DNA, 26 bp, Artificial Sequence
  antisense primer for hsa-miR26b-5p
ggtccagtttttttttttttttacct

SEQ ID NO: 28 - DNA, 19 bp, Artificial Sequence
  sense primer for hsa-miR107-5p
gcagagcagcattgtacag

SEQ ID NO: 29 - DNA, 27 bp, Artificial Sequence
  antisense primer for hsa-miR107-5p
ggtccagtttttttttttttttgatag

SEQ ID NO: 30 - DNA, 17 bp, Artificial Sequence
  sense primer for hsa-miR125b-5p
gcagtccctgagaccct

SEQ ID NO: 31 - DNA, 26 bp, Artificial Sequence
  antisense primer for hsa-miR125b-5p
ccagtttttttttttttttcacaagt

SEQ ID NO: 32 - DNA, 19 bp, Artificial Sequence
  sense primer for hsa-miR194-5p
cagtgtaacagcaactcca

SEQ ID NO: 33 - DNA, 26 bp, Artificial Sequence
  antisense primer for hsa-miR194-5p
tccagtttttttttttttttccacat

SEQ ID NO: 34 - DNA, 18 bp, Artificial Sequence
  sense primer for hsa-miR222-3p
gcagagctacatctggct

SEQ ID NO: 35 - DNA, 26 bp, Artificial Sequence
  antisense primer for hsa-miR222-3p
ccagtttttttttttttttacccagt

SEQ ID NO: 36 - DNA, 17 bp, Artificial Sequence
  sense primer for hsa-miR423-5p
cagtgaggggcagagag

SEQ ID NO: 37 - DNA, 28 bp, Artificial Sequence
  antisense primer for hsa-miR423-5p
ggtccagtttttttttttttttaaagtc

SEQ ID NO: 38 - DNA, 18 bp, Artificial Sequence
  sense primer for hsa-miR424-5p
agcagcagcaattcatgt

SEQ ID NO: 39 - DNA, 26 bp, Artificial Sequence
  antisense primer for hsa-miR424-5p
aggtccagtttttttttttttttcaa

SEQ ID NO: 40 - DNA, 20 bp, Artificial Sequence
  sense primer for hsa-miR660-5p
agtacccattgcatatcgga

SEQ ID NO: 41 - DNA, 26 bp, Artificial Sequence
  antisense primer for hsa-miR660-5p
ggtccagtttttttttttttttcaac

SEQ ID NO: 42 - DNA, 19 bp, Artificial Sequence
  sense primer for hsa-let7a-5p
gcagtgaggtagtaggttg

SEQ ID NO: 43 - DNA, 30 bp, Artificial Sequence
  antisense primer for hsa-let7a-5p
ggtccagtttttttttttttttaactatac

SEQ ID NO: 44 - DNA, 20 bp, Artificial Sequence
  sense primer for hsa-let7d-5p
cgcagagaggtagtaggttg

SEQ ID NO: 45 - DNA, 29 bp, Artificial Sequence
  antisense primer for hsa-let7d-5p
ggtccagtttttttttttttttaactatg

SEQ ID NO: 46 - DNA, 19 bp, Artificial Sequence
  sense primer for hsa-let7e-5p
gcagtgaggtaggaggttg

SEQ ID NO: 47 - DNA, 30 bp, Artificial Sequence; identical to SEQ ID NO: 43
  antisense primer for hsa-let7e-5p

SEQ ID NO: 48 - DNA, 20 bp, Artificial Sequence
  sense primer for hsa-let7f-5p
cgcagtgaggtagtagattg

SEQ ID NO: 49 - DNA, 27 bp, Artificial Sequence
  antisense primer for hsa-let7f-5p
caggtccagtttttttttttttttaac

SEQ ID NO: 50 - DNA, 21 bp, Artificial Sequence
  sense primer for hsa-let7i-5p
gcagtgaggtagtagtttgtg

SEQ ID NO: 51 - DNA, 27 bp, Artificial Sequence
  antisense primer for hsa-let7i-5p
ggtccagtttttttttttttttaacag

SEQ ID NO: 52 - DNA, 26 bp, Artificial Sequence
  universal primer for reverse transcription (RT) reaction
  misc_feature (26)..(26): n is a, c, g, or t
caggtccagtttttttttttttttvn